European Patent Application EP 4 722 243 A1, published April 8, 2026. Title: 结合IL-11的抗体、其抗原结合片段及其用途. Applicant: 北京东方百泰生物科技股份有限公司. The sequence listing filed with the application follows.

SEQUENCE LISTING (40 sequences)

SEQ ID NO: 1 - protein, 5 aa, synthetic construct
DYYMF

SEQ ID NO: 2 - protein, 17 aa, synthetic construct
TISDGGTYTYYPDSVKG

SEQ ID NO: 3 - protein, 13 aa, synthetic construct
DGGYVSSPEAMDY

SEQ ID NO: 4 - protein, 11 aa, synthetic construct
RASQDISNYLN

SEQ ID NO: 5 - protein, 7 aa, synthetic construct
YTSRLHS

SEQ ID NO: 6 - protein, 9 aa, synthetic construct
QQGNTLPPT

SEQ ID NO: 7 - protein, 9 aa, synthetic construct
QQGNTLPWT

SEQ ID NO: 8 - protein, 5 aa, synthetic construct
SYWMH

SEQ ID NO: 9 - protein, 17 aa, synthetic construct
VIDPSDSYTTYNQKFKG

SEQ ID NO: 10 - protein, 11 aa, synthetic construct
YGYDVNWYFDV

SEQ ID NO: 11 - protein, 16 aa, synthetic construct
RSSQSIVHSNGNTYLE

SEQ ID NO: 12 - protein, 7 aa, synthetic construct
EVSNRFS

SEQ ID NO: 13 - protein, 9 aa, synthetic construct
FQGSHVPWT

SEQ ID NO: 14 - protein, 17 aa, synthetic construct
TISDGGSYSYYPDSVKG

SEQ ID NO: 15 - protein, 13 aa, synthetic construct
DGGYISSPEAMDY

SEQ ID NO: 16 - protein, 122 aa, synthetic construct
EVKLEESGGGLVKPGGSLKLSCAASGFTFSDYYMFWVRQTPEKRLEWVATISDGGTYTYYPDSVKGRFTISRDNAKNNLYLQMTSLKSEDTAMYYCARDGGYVSSPEAMDYWGQGTSVTVSS

SEQ ID NO: 17 - protein, 107 aa, synthetic construct
DIVLTQSTSSLSASLGDRVTISCRASQDISNYLNWYQQKPDGTVKLLIYYTSRLHSGVPSRFSGSGSGTDYSLTISNLEQEDIATYFCQQGNTLPPTFGGGTKLEIK

SEQ ID NO: 18 - protein, 107 aa, synthetic construct
DIVLTQSTSSLSASLGDRVTISCRASQDISNYLNWYQQKPDGTVKLLIYYTSRLHSGVPSRFSGSGSGTDYSLTISNLEQEDIATYFCQQGNTLPWTFGGGTKLEIK

SEQ ID NO: 19 - protein, 120 aa, synthetic construct
EVKLEQSGAEVVKPGALVKMSCKASGYTFTSYWMHWVKQRPGQGLEWIGVIDPSDSYTTYNQKFKGKATLTVDTSSSTGYMQLSSLTSEDSAVYYCSQYGYDVNWYFDVWGAGTTVTVSS

SEQ ID NO: 20 - protein, 112 aa, synthetic construct
DIVMTQTTLSLPVSLGDQASISCRSSQSIVHSNGNTYLEWYLQKPGQSPKLLIYEVSNRFSGVPDRFSGSGSGTDFTLKISRVEAEDLGVYYCFQGSHVPWTFGGGTKLEIK

SEQ ID NO: 21 - protein, 122 aa, synthetic construct
EVQLEESGGGLVKPGGSLKLSCVASGFTFSDYYMFWVRQTPEKRLEWVATISDGGSYSYYPDSVKGRFTISRDNAKNNLYLQMSSLRSEDTAMYYCARDGGYISSPEAMDYWGQGTSVTVSS

SEQ ID NO: 22 - protein, 106 aa, synthetic construct
ADAAPTVSIFPPSSEQLTSGGASVVCFLNNFYPKDINVKWKIDGSERQNGVLNSWTDQDSKDSTYSMSSTLTLTKDEYERHNSYTCEATHKTSTSPIVKSFNRNEC

SEQ ID NO: 23 - protein, 323 aa, synthetic construct
AKTTPPSVYPLAPGSAAQTNSMVTLGCLVKGYFPEPVTVTWNSGSLSSGVHTFPAVLQSDLYTLSSSVTVPSSTWPSETVTCNVAHPASSTKVDKKIVPRDCGCKPCICTVPEVSSVFIFPPKPKDVLTITLTPKVTCVVVDISKDDPEVQFSWFVDDVEVHTAQTQPREEQFNSTFRSVSELPIMHQDWLNGKEFKCRVNSAAFPAPIEKTISKTKGRPKAPQVYTIPPPKEQMAKDKVSLTCMITDFFPEDITVEWQWNGQPAENYKNTQPIMDTDGSYFVYSKLNVQKSNWEAGNTFTCSVLHEGLHNHHTEKSLSHSPG

SEQ ID NO: 24 - protein, 330 aa, synthetic construct
AKTTAPSVYPLAPVCGDTTGSSVTLGCLVKGYFPEPVTLTWNSGSLSSGVHTFPAVLQSDLYTLSSSVTVTSSTWPSQSITCNVAHPASSTKVDKKIEPRGPTIKPCPPCKCPAPNLLGGPSVFIFPPKIKDVLMISLSPIVTCVVVDVSEDDPDVQISWFVNNVEVHTAQTQTHREDYNSTLRVVSALPIQHQDWMSGKEFKCKVNNKDLPAPIERTISKPKGSVRAPQVYVLPPPEEEMTKKQVTLTCMVTDFMPEDIYVEWTNNGKTELNYKNTEPVLDSDGSYFMYSKLRVEKKNWVERNSYSCSVVHEGLHNHHTTKSFSRTPGK

SEQ ID NO: 25 - protein, 336 aa, synthetic construct
AKTTPPSVYPLAPGCGDTTGSSVTLGCLVKGYFPESVTVTWNSGSLSSSVHTFPALLQSGLYTMSSSVTVPSSTWPSQTVTCSVAHPASSTTVDKKLEPSGPISTINPCPPCKECHKCPAPNLEGGPSVFIFPPNIKDVLMISLTPKVTCVVVDVSEDDPDVQISWFVNNVEVHTAQTQTHREDYNSTIRVVSTLPIQHQDWMSGKEFKCKVNNKDLPSPIERTISKIKGLVRAPQVYILPPPAEQLSRKDVSLTCLVVGFNPGDISVEWTSNGHTEENYKDTAPVLDSDGSYFIYSKLNMKTSKWEKTDSFSCNVRHEGLKNYYLKKTISRSPGK

SEQ ID NO: 26 - protein, 399 aa, synthetic construct
ATTTAPSVYPLVPGCSDTSGSSVTLGCLVKGYFPEPVTVKWNYGALSSGVRTVSSVLQSGFYSLSSLVTVPSSTWPSQTVICNVAHPASKTELIKRIEPRIPKPSTPPGSSCPPGNILGGPSVFIFPPKPKDALMISLTPKVTCVVVDVSEDDPDVHVSWFVDNKEVHTAWTQPREAQYNSTFRVVSALPIQHQDWMRGKEFKCKVNNKALPAPIERTISKPKGRAQTPQVYTIPPPREQMSKKKVSLTCLVTNFFSEAISVEWERNGELEQDYKNTPPILDSDGTYFLYSKLTVDTDSWLQGEIFTCSVVHEALHNHHTQKNLSRSPELELNETCAEAQDGELDGLWTTITIFISLFLLSVCYSASVTLFKVKWIFSSVVQVKQTAIPDYRNMIGQGA

SEQ ID NO: 27 - protein, 330 aa, synthetic construct
ASTKGPSVFPLAPSSKSTSGGTAALGCLVKDYFPEPVTVSWNSGALTSGVHTFPAVLQSSGLYSLSSVVTVPSSSLGTQTYICNVNHKPSNTKVDKRVEPKSCDKTHTCPPCPAPEAAGGPSVFLFPPKPKDTLMISRTPEVTCVVVDVSHEDPEVKFNWYVDGVEVHNAKTKPREEQYNSTYRVVSVLTVLHQDWLNGKEYKCKVSNKALPAPIEKTISKAKGQPREPQVYTLPPSREEMTKNQVSLTCLVKGFYPSDIAVEWESNGQPENNYKTTPPVLDSDGSFFLYSKLTVDKSRWQQGNVFSCSVMHEALHNHYTQKSLSLSPGK

SEQ ID NO: 28 - protein, 326 aa, synthetic construct
ASTKGPSVFPLAPCSRSTSESTAALGCLVKDYFPEPVTVSWNSGALTSGVHTFPAVLQSSGLYSLSSVVTVPSSNFGTQTYTCNVDHKPSNTKVDKTVERKCCVECPPCPAPPVAGPSVFLFPPKPKDTLMISRTPEVTCVVVDVSHEDPEVQFNWYVDGVEVHNAKTKPREEQFNSTFRVVSVLTVVHQDWLNGKEYKCKVSNKGLPAPIEKTISKTKGQPREPQVYTLPPSREEMTKNQVSLTCLVKGFYPSDIAVEWESNGQPENNYKTTPPMLDSDGSFFLYSKLTVDKSRWQQGNVFSCSVMHEALHNHYTQKSLSLSPGK

SEQ ID NO: 29 - protein, 327 aa, synthetic construct
ASTKGPSVFPLAPCSRSTSESTAALGCLVKDYFPEPVTVSWNSGALTSGVHTFPAVLQSSGLYSLSSVVTVPSSSLGTKTYTCNVDHKPSNTKVDKRVESKYGPPCPPCPAPEFLGGPSVFLFPPKPKDTLMISRTPEVTCVVVDVSQEDPEVQFNWYVDGVEVHNAKTKPREEQFNSTYRVVSVLTVLHQDWLNGKEYKCKVSNKGLPSSIEKTISKAKGQPREPQVYTLPPSQEEMTKNQVSLTCLVKGFYPSDIAVEWESNGQPENNYKTTPPVLDSDGSFFLYSRLTVDKSRWQEGNVFSCSVMHEALHNHYTQKSLSLSLGK

SEQ ID NO: 30 - protein, 107 aa, synthetic construct [sequence omitted]

SEQ ID NO: 31 - protein, 122 aa, synthetic construct
QVQLVESGGGLVKPGGSLRLSCAASGFTFSDYYMFWVRQAPGKGLEWVATISDGGTYTYYPDSVKGRFTISRDNAKNSLYLQMNSLRAEDTAVYYCARDGGYVSSPEAMDYWGQGTLVTVSS

SEQ ID NO: 32 - protein, 107 aa, synthetic construct
DIVLTQSPSSLSASVGDRVTITCRASQDISNYLNWYQQKPGKAPKLLIYYTSRLHSGVPSRFSGSGSGTDFTFTISSLQPEDIATYYCQQGNTLPPTFGGGTKVEIK

SEQ ID NO: 33 - protein, 122 aa, synthetic construct
QVQLVESGGGLVKPGGSLRLSCAASGFTFSDYYMFWVRQAPGKGLEWVSTISDGGTYTYYPDSVKGRFTISRDNAKNSLYLQMNSLRAEDTAVYYCARDGGYVSSPEAMDYWGQGTLVTVSS

SEQ ID NO: 34 - protein, 107 aa, synthetic construct
DIVLTQSPSSLSASVGDRVTITCRASQDISNYLNWYQQKPGKAPKLLIYYTSRLHSGVPSRFSGSGSGTDYTFTISSLQPEDIATYYCQQGNTLPPTFGGGTKVEIK

SEQ ID NO: 35 - protein, 107 aa, synthetic construct
DIVLTQSPSSLSASVGDRVTITCRASQDISNYLNWYQQKPGKAVKLLIYYTSRLHSGVPSRFSGSGSGTDYTFTISSLQPEDIATYFCQQGNTLPPTFGGGTKVEIK

SEQ ID NO: 36 - protein, 122 aa, synthetic construct
QVQLVESGGGLVKPGGSLRLSCAASGFTFSDYYMFWVRQAPGKGLEWVATISDGGTYTYYPDSVKGRFTISRDNAKNSLYLQMNSLRAEDTAMYYCARDGGYVSSPEAMDYWGQGTSVTVSS

SEQ ID NO: 37 - protein, 107 aa, synthetic construct
DIVLTQSPSSLSASVGDRVTITCRASQDISNYLNWYQQKPGGAVKLLIYYTSRLHSGVPSRFSGSGSGTDYTFTISSLQPEDIATYFCQQGNTLPPTFGGGTKVEIK

SEQ ID NO: 38 - protein, 107 aa, synthetic construct
DIVLTQSPSSLSASVGDRVTITCRASQDISNYLNWYQQKPGKAPKLLIYYTSRLHSGVPSRFSGSGSGTDFTFTISSLQPEDIATYYCQQGNTLPWTFGGGTKVEIK

SEQ ID NO: 39 - protein, 107 aa, synthetic construct
DIVLTQSPSSLSASVGDRVTITCRASQDISNYLNWYQQKPGKAPKLLIYYTSRLHSGVPSRFSGSGSGTDYTFTISSLQPEDIATYYCQQGNTLPWTFGGGTKVEIK

SEQ ID NO: 40 - protein, 107 aa, synthetic construct
DIVLTQSPSSLSASVGDRVTITCRASQDISNYLNWYQQKPGGTVKLLIYYTSRLHSGVPSRFSGSGSGTDYTFTISSLQPEDIATYFCQQGNTLPWTFGGGTKVEIK